European Patent Specification EP 3 250 681 B1, published May 3, 2023. Title: COMPOSITIONS AND METHODS FOR T CELL DELIVERY OF THERAPEUTIC MOLECULES. Applicant: The Trustees of the University of Pennsylvania Zhao, Yangbing Liu, Xiaojun June, Carl H. The sequence listing filed with the application follows.

SEQUENCE LISTING (17 sequences)

SEQ ID NO: 1 - DNA, 717 bp, Homo Sapiens
atggaggcggcggtcgctgctccgcgtccccggctgctcctcctcgtgctggcggcggcggcggcggcggcggcggcgctgctcccgggggcgacggcgttacagtgtttctgccacctctgtacaaaagacaattttacttgtgtgacagatgggctctgctttgtctctgtcacagagaccacagacaaagttatacacaacagcatgtgtatagctgaaattgacttaattcctcgagataggccgtttgtatgtgcaccctcttcaaaaactgggtctgtgactacaacatattgctgcaatcaggaccattgcaataaaatagaacttccaactactgtaaagtcatcacctggccttggtcctgtggaactggcagctgtcattgctggaccagtgtgcttcgtctgcatctcactcatgttgatggtctatatcagggccgcacggcacctgtgcccgccgctgcccacaccctgtgccagctccgccattgagttccctggagggaaggagacttggcagtggatcaacccagtggacttccaggaagaggcatccctgcaggaggccctggtggtagagatgtcctgggacaaaggcgagaggactgagcctctcgagaagacagagctacctgagggtgcccctgagctggccctggatacagagttgtccttggaggatggagacaggtgcaaggccaagatgtga

SEQ ID NO: 2 - DNA, 1212 bp, Homo Sapiens
atgggtcgggggctgctcaggggcctgtggccgctgcacatcgtcctgtggacgcgtatcgccagcacgatcccaccgcacgttcagaagtcggttaataacgacatgatagtcactgacaacaacggtgcagtcaagtttccacaactgtgtaaattttgtgatgtgagattttccacctgtgacaaccagaaatcctgcatgagcaactgcagcatcacctccatctgtgagaagccacaggaagtctgtgtggctgtatggagaaagaatgacgagaacataacactagagacagtttgccatgaccccaagctcccctaccatgactttattctggaagatgctgcttctccaaagtgcattatgaaggaaaaaaaaaagcctggtgagactttcttcatgtgttcctgtagctctgatgagtgcaatgacaacatcatcttctcagaagaatataacaccagcaatcctgacttgttgctagtcatatttcaagtgacaggcatcagcctcctgccaccactgggagttgccatatctgtcatcatcatcttctaccagcaaaaggtgtttgttctcctagcagccctcagacctcagtggtgtagcagagaaattccagatccagcaaatagcacttgcgctaagaaatatcccattgcagaggagaagacacagctgcccttggacaggctcctgatagactggcccacgcctgaagatcctgaaccgctggtcatcagtgaagtccttcatcaagtgaccccagttttcagacatcccccctgctccaactggccacaaagggaaaaaggaatccaaggtcatcaggcctctgagaaagacatgatgcacagtgcctcaagcccaccacctccaagagctctccaagctgagagcagacaactggtggatctgtacaaggtgctggagagcaggggctccgacccaaagccagaaaacccagcctgtccctggacggtgctcccagcaggtgaccttcccacccatgatggctacttaccctccaacatagatgacctcccctcacatgaggcacctctcgctgactctctggaagaactggagcctcagcacatctccctttctgttttcccctcaagttctcttcacccactcaccttctcctgtggtgataagctgactctggatcagttaaagatgaggtgtgactccctcatgctctga

SEQ ID NO: 3 - DNA, 1515 bp, Homo Sapiens
atgggttggtcctgcatcatcctgtttctcgtggccaccgccaccggcgtgcactccgaaattgtgttgacacagtctccagccaccctgtctttgtctccaggggaaagagccaccctctcctgcagggccagtcagagtgttcgcagctacttagcctggtaccaacagaaacctggccaggctcccaggctcctcatctatgatgcatccaacagggccactggcatcccagccaggttcagtggcagtgggtctgggacagacttcactctcaccatcagcagcctagagcctgaagattttgcagtttattactgtcagcagcgtagcaactggcctccgacgttcggccaagggaccaaggtggaaatcaaaagtggagggggcggttcacagctgcaggtgcaggagtcgggcccaggactggtgaagccttcggagaccctgtccctcacctgcactgtctctggtggctccatcagcaacagttatttctcctggggctggatccgccagcccccagggaagggactggagtggattgggagtttctattatggtgaaaaaacctactacaacccgtccctcaagagccgagccaccatatccattgacacgtccaagagccagttctccctgaagctgagctctgtgaccgccgcagacacggctgtgtattactgtccgagagggcctactatgattcggggagttatagactcctggggccagggaaccctggtgacggtgtcgtcggggggcggggggagtcaggtgcagctggtgcagtccggagccgaggtaaagaagccaggcgcttccgtcaaggtgtcatgcaaggcctcaggctacaccttcacaagctattacatccactgggtgcgccaagctcccggtcagggcttggagtggatcgggtgcatttacccagggaacgtcaacacaaactacaacgagaagttcaaggatcgggcaaccctgaccgtggacacatccatctctaccgcctacatggagctgtcacgcctgcgctctgatgacaccgcagtgtacttctgtaccaggagtcactacggcctggactggaactttgatgtctggggccagggaaccaccgtgacggtgtccagtgtggagggcggtagtggcggctctggtgggtccggaggctcaggcggcgtgatggatgacattcagatgacccagagtccctcctccctctccgcttccgtcggagaccgcgtgaccatcacttgtcacgcctcacagaatatctacgtgtggctgaactggtaccaacagaagcccggcaaggcccccaagctgcttatctataaagcgtccaacctccacacgggagtcccttcccgcttctccggatccggcagtgggacggacttcacactcacaatctcgtcgctgcagccagaggactttgcgacgtactactgccagcagggccagacctacccatatactttcggcggcgggaccaaggtggagattaagtaa

SEQ ID NO: 4 - DNA, 1515 bp, Homo Sapiens
atgggttggtcctgcatcatcctgtttctcgtggccaccgccaccggcgtgcactccgaaattgtgttgacacagtctccagccaccctgtctttgtctccaggggaaagagccaccctctcctgcagggccagtcagagtgttagaagtttcttagcctggtaccaacagaaacctggccaggctcccaggctcctcatctatgatgcatccaacagggccactggcatcccagccaggttcagtggcagtggggtctgggacagacttcactctcaccatcagcagcctagagcctgaagattttgcagtttattactgtcagcagcgtagcaactggcctccgacgttcggccaagggaccaaggtggaaatcaaaagtggagggggcggttcacagctacagctgcaggagtcgggcccaggactggtgaagccttcggagaccctatccctcacctgcactgtctctggtggctccatcagcagtagtagttactcctggggctggatccgccagcccccagggaagggcctggagtggattggagtttctattacagtgggatcacctactacagcccgtccctcaagagtcgaattatcatatccgaagacacgtccaagaaccagttctccctgaagctgagttctgtgaccgccgcagacacggctgtgtattactgtgcgagcgggtttactatgattcggggagcccttgactactggggccagggaaccctggtgacggtgtcgtcggggggcggggggagtcaggtgcagctggtgcagtccggagccgaggtaaagaagccaggcgcttccgtcaaggtgtcatgcaaggcctcaggctacaccttcacaagctattacatccactgggtgcgccaagctcccggtcagggcttggagtggatcgggtgcatttacccagggaacgtcaacacaaactacaacgagaagttcaaggatcgggcaaccctgaccgtggacacatccatctctaccgcctacatggagctgtcacgcctgcgctctgatgacaccgcagtgtacttctgtaccaggagtcactacggcctggactggaactttgatgtctggggccagggaaccaccgtgacggtgtccagtgtggagggcggtagtggcggctctggtgggtccggaggctcaggcggcgtgatggatgacattcagatgacccagagtccctcctccctctccgcttccgtcggagaccgcgtgaccatcacttgtcacgcctcacagaatatctacgtgtggctgaactggtaccaacagaagcccggcaaggcccccaagctgcttatctataaagcgtccaacctccacacgggagtcccttcccgcttctccggatccggcagtgggacggacttcacactcacaatctcgtcgctgcagccagaggactttgcgacgtactactgccagcagggccagacctacccatatactttcggcggcgggaccaaggtggagattaagtaa

SEQ ID NO: 5 - DNA, 1449 bp, Homo Sapiens
atggatccccagtgcactatgggactgagtaacattctctttgtgatggccttcctgctctctggtgctgctcctctgaagattcaagcttatttcaatgagactgcagacctgccatgccaatttgcaaactctcaaaaccaaagcctgagtgagctagtagtattttggcaggaccaggaaaacttggttctgaatgaggtatacttaggcaaagagaaatttgacagtgttcattccaagtatatgggccgcacaagttttgattcggacagttggaccctgagacttcacaatcttcagatcaaggacaagggcttgtatcaatgtatcatccatcacaaaaagcccacaggaatgattcgcatccaccagatgaattctgaactgtcagtgcttgctaacttcagtcaacctgaaatagtaccaatttctaatataacagaaaatgtgtacataaatttgacctgctcatctatacacggttacccagaacctaagaagatgagtgttttgctaagaaccaagaattcaactatcgagtatgatggtattatgcagaaatctcaagataatgtcacagaactgtacgacgtttccatcagcttgtctgtttcattccctgatgttacgagcaatatgaccatcttctgtattctggaaactgacaagacgcggcttttatcttcacctttctctatagagcttgaggaccctcagcctcccccagaccacattcctggcggagggggaagtggcgggggtgggtccggcggcggcggctcgtttactgtcacggttcccaaggacctatatgtggtagagtatggtagcaatatgacaattgaatgcaaattcccagtagaaaaacaattagacctggctgcactaattgtctattgggaaatggaggataagaacattattcaatttgtgcatggagaggaagacctgaaggttcagcatagtagctacagacagagggcccggctgttgaaggaccagctctccctgggaaatgctgcacttcagatcacagatgtgaaattgcaggatgcaggggtgtaccgctgcatgatcagctatggtggtgccgactacaagcgaattactgtgaaagtcaatgccccatacaacaaaatcaaccaaagaattttggttgtggatccagtcacctctgaacatgaactgacatgtcaggctgagggctaccccaaggccgaagtcatctggacaagcagtgaccatcaagtcctgagtggtaagaccaccaccaccaattccaagagagaggagaagcttttcaatgtgaccagcacactgagaatcaacacaacaactaatgagattttctactgcacttttaggagattagatcctgaggaaaaccatacagctgaattggtcatcccagaactacctctggcacatcctccaaatgaaaggtaa

SEQ ID NO: 6 - DNA, 1392 bp, Homo Sapiens
atggatccccagtgcactatgggactgagtaacattctctttgtgatggccttcctgctctctggtgctgctcctctgaagattcaagcttatttcaatgagactgcagacctgccatgccaatttgcaaactctcaaaaccaaagcctgagtgagctagtagtattttggcaggaccaggaaaacttggttctgaatgaggtatacttaggcaaagagaaatttgacagtgttcattccaagtatatgggccgcacaagttttgattcggacagttggaccctgagacttcacaatcttcagatcaaggacaagggcttgtatcaatgtatcatccatcacaaaaagcccacaggaatgattcgcatccaccagatgaattctgaactgtcagtgcttgctaacttcagtcaacctgaaatagtaccaatttctaatataacagaaaatgtgtacataaatttgacctgctcatctatacacggttacccagaacctaagaagatgagtgttttgctaagaaccaagaattcaactatcgagtatgatggtattatgcagaaatctcaagataatgtcacagaactgtacgacgtttccatcagcttgtctgtttcattccctgatgttacgagcaatatgaccatcttctgtattctggaaactgacaagacgcggcttttatcttcacctttctctatagagcttgaggaccctcagcctcccccagaccacattcctggcggagggggaagtggcgggggtgggtccggcggcggcggctcgttattcacagtgacagtccctaaggaactgtacataatagagcatggcagcaatgtgaccctggaatgcaactttgacactggaagtcatgtgaaccttggagcaataacagccagtttgcaaaaggtggaaaatgatacatccccacaccgtgaaagagccactttgctggaggagcagctgcccctagggaaggcctcgttccacatacctcaagtccaagtgagggacgaaggacagtaccaatgcataatcatctatggggtcgcctgggactacaagtacctgactctgaaagtcaaagcttcctacaggaaaataaacactcacatcctaaaggttccagaaacagatgaggtagagctcacctgccaggctacaggttatcctctggcagaagtatcctggccaaacgtcagcgttcctgccaacaccagccactccaggacccctgaaggcctctaccaggtcaccagtgttctgcgcctaaagccaccccctggcagaaacttcagctgtgtgttctggaatactcacgtgagggaacttactttggccagcattgaccttcaaagtcagatggaacccaggacccatccaacttaa

SEQ ID NO: 7 - DNA, 1434 bp, Homo Sapiens
atgggccacacacggaggcagggaacatcaccatccaagtgtccatacctcaatttctttcagctcttggtgctggctggtctttctcacttctgttcaggtgttatccacgtgaccaaggaagtgaaagaagtggcaacgctgtcctgtggtcacaatgtttctgttgaagagctggcacaaactcgcatctactggcaaaaggagaagaaaatggtgctgactatgatgtctggggacatgaatatatggcccgagtacaagaaccggaccatctttgatatcactaataacctctccattgtgatcctggctctgcgcccatctgacgagggcacatacgagtgtgttgttctgaagtatgaaaaagacgctttcaagcgggaacacctggctgaagtgacgttatcagtcaaagctgacttccctacacctagtatatctgactttgaaattccaacttctaatattagaaggataatttgctcaacctctggaggttttccagagcctcacctctcctggttggaaaatggagaagaattaaatgccatcaacacaacagtttcccaagatcctgaaactgagctctatgctgttagcagcaaactggatttcaatatgacaaccaaccacagcttcatgtgtctcatcaagtatggacatttaagagtgaatcagaccttcaactggaatacaaccaagcaagagcattttcctgataacggcggagggggaagtggcgggggtgggtccggcggcggcggctcgtttactgtcacggttcccaaggacctatatgtggtagagtatggtagcaatatgacaattgaatgcaaattcccagtagaaaaacaattagacctggctgcactaattgtctattgggaaatggaggataagaacattattcaatttgtgcatggagaggaagacctgaaggttcagcatagtagctacagacagagggcccggctgttgaaggaccagctctccctgggaaatgctgcacttcagatcacagatgtgaaattgcaggatgcaggggtgtaccgctgcatgatcagctatggtggtgccgactacaagcgaattactgtgaaagtcaatgccccatacaacaaaatcaaccaaagaattttggttgtggatccagtcacctctgaacatgaactgacatgtcaggctgagggctaccccaaggccgaagtcatctggacaagcagtgaccatcaagtcctgagtggtaagaccaccaccaccaattccaagagagaggagaagcttttcaatgtgaccagcacactgagaatcaacacaacaactaatgagattttctactgcacttttaggagattagatcctgaggaaaaccatacagctgaattggtcatcccagaactacctctggcacatcctccaaatgaaaggtaa

SEQ ID NO: 8 - DNA, 1377 bp, Homo Sapiens
atgggccacacacggaggcagggaacatcaccatccaagtgtccatacctcaatttctttcagctcttggtgctggctggtctttctcacttctgttcaggtgttatccacgtgaccaaggaagtgaaagaagtggcaacgctgtcctgtggtcacaatgtttctgttgaagagctggcacaaactcgcatctactggcaaaaggagaagaaaatggtgctgactatgatgtctggggacatgaatatatggcccgagtacaagaaccggaccatctttgatatcactaataacctctccattgtgatcctggctctgcgcccatctgacgagggcacatacgagtgtgttgttctgaagtatgaaaaagacgctttcaagcgggaacacctggctgaagtgacgttatcagtcaaagctgacttccctacacctagtatatctgactttgaaattccaacttctaatattagaaggataatttgctcaacctctggaggttttccagagcctcacctctcctggttggaaaatggagaagaattaaatgccatcaacacaacagtttcccaagatcctgaaactgagctctatgctgttagcagcaaactggatttcaatatgacaaccaaccacagcttcatgtgtctcatcaagtatggacatttaagagtgaatcagaccttcaactggaatacaaccaagcaagagcattttcctgataacggcggagggggaagtggcgggggtgggtccggcggcggcggctcgttattcacagtgacagtccctaaggaactgtacataatagagcatggcagcaatgtgaccctggaatgcaactttgacactggaagtcatgtgaaccttggagcaataacagccagtttgcaaaaggtggaaaatgatacatccccacaccgtgaaagagccactttgctggaggagcagctgcccctagggaaggcctcgttccacatacctcaagtccaagtgagggacgaaggacagtaccaatgcataatcatctatggggtcgcctgggactacaagtacctgactctgaaagtcaaagcttcctacaggaaaataaacactcacatcctaaaggttccagaaacagatgaggtagagctcacctgccaggctacaggttatcctctggcagaagtatcctggccaaacgtcagcgttcctgccaacaccagccactccaggacccctgaaggcctctaccaggtcaccagtgttctgcgcctaaagccaccccctggcagaaacttcagctgtgtgttctggaatactcacgtgagggaacttactttggccagcattgaccttcaaagtcagatggaacccaggacccatccaacttaa

SEQ ID NO: 9 - DNA, 1440 bp, Homo Sapiens
atgaggatatttgctgtctttatattcatgacctactggcatttgctgaacgcatttactgtcacggttcccaaggacctatatgtggtagagtatggtagcaatatgacaattgaatgcaaattcccagtagaaaaacaattagacctggctgcactaattgtctattgggaaatggaggataagaacattattcaatttgtgcatggagaggaagacctgaaggttcagcatagtagctacagacagagggcccggctgttgaaggaccagctctccctgggaaatgctgcacttcagatcacagatgtgaaattgcaggatgcaggggtgtaccgctgcatgatcagctatggtggtgccgactacaagcgaattactgtgaaagtcaatgccccatacaacaaaatcaaccaaagaattttggttgtggatccagtcacctctgaacatgaactgacatgtcaggctgagggctaccccaaggccgaagtcatctggacaagcagtgaccatcaagtcctgagtggtaagaccaccaccaccaattccaagagagaggagaagcttttcaatgtgaccagcacactgagaatcaacacaacaactaatgagattttctactgcacttttaggagattagatcctgaggaaaaccatacagctgaattggtcatcccagaactacctctggcacatcctccaaatgaaaggggcggagggggaagtggcgggggtgggtccggcggcggcggctcgggtgctgctcctctgaagattcaagcttatttcaatgagactgcagacctgccatgccaatttgcaaactctcaaaaccaaagcctgagtgagctagtagtattttggcaggaccaggaaaacttggttctgaatgaggtatacttaggcaaagagaaatttgacagtgttcattccaagtatatgggccgcacaagttttgattcggacagttggaccctgagacttcacaatcttcagatcaaggacaagggcttgtatcaatgtatcatccatcacaaaaagcccacaggaatgattcgcatccaccagatgaattctgaactgtcagtgcttgctaacttcagtcaacctgaaatagtaccaatttctaatataacagaaaatgtgtacataaatttgacctgctcatctatacacggttacccagaacctaagaagatgagtgttttgctaagaaccaagaattcaactatcgagtatgatggtattatgcagaaatctcaagataatgtcacagaactgtacgacgtttccatcagcttgtctgtttcattccctgatgttacgagcaatatgaccatcttctgtattctggaaactgacaagacgcggcttttatcttcacctttctctatagagcttgaggaccctcagcctcccccagaccacattccttaa

SEQ ID NO: 10 - DNA, 1408 bp, Homo Sapiens
atgaggatatttgctgtctttatattcatgacctactggcatttgctgaacgcatttactgtcacggttcccaaggacctatatgtggtagagtatggtagcaatatgacaattgaatgcaaattcccagtagaaaaacaattagacctggctgcactaattgtctattgggaaatggaggataagaacattattcaatttgtgcatggagaggaagacctgaaggttcagcatagtagctacagacagagggcccggctgttgaaggaccagctctccctgggaaatgctgcacttcagatcacagatgtgaaattgcaggatgcaggggtgtaccgctgcatgatcagctatggtggtgccgactacaagcgaattactgtgaaagtcaatgccccatacaacaaaatcaaccaaagaattttggttgtggatccagtcacctctgaacatgaactgacatgtcaggctgagggctaccccaaggccgaagtcatctggacaagcagtgaccatcaagtcctgagtggtaagaccaccaccaccaattccaagagagaggagaagcttttcaatgtgaccagcacactgagaatcaacacaacaactaatgagattttctactgcacttttaggagattagatcctgaggaaaaccatacagctgaattggtcatcccagaactacctctggcacatcctccaaatgaaaggggcggagggggaagtggcgggggtgggtccggcggcggcggctcgtctttctcacttctgttcaggtgttatccacgtgaccaaggaagtgaaagaagtggcaacgctgtcctgtggtcacaatgtttctgttgaagagctggcacaaactcgcatctactggcaaaaggagaagaaaatggtgctgactatgatgtctggggacatgaatatatggcccgagtacaagaaccggaccatctttgatatcactaataacctctccattgtgatcctggctctgcgcccatctgacgagggcacatacgagtgtgttgttctgaagtatgaaaaagacgctttcaagcgggaacacctggctgaagtgacgttatcagtcaaagctgacttccctacacctagtatatctgactttgaaattccaacttctaatattagaaggataatttgctcaacctctggaggttttccagagcctcacctctcctggttggaaaatggagaagaattaaatgccatcaacacaacagtttcccaagatcctgaaactgagctctatgctgttagcagcaaactggatttcaatatgacaaccaaccacagcttcatgtgtctcatcaagtatggacatttaagagtgaatcagaccttcaactggaatacaaccaagcaagagcattttcctgataactaa

SEQ ID NO: 11 - DNA, 1383 bp, Homo Sapiens
atgatcttcctcctgctaatgttgagcctggaattgcagcttcaccagatagcagctttattcacagtgacagtccctaaggaactgtacataatagagcatggcagcaatgtgaccctggaatgcaactttgacactggaagtcatgtgaaccttggagcaataacagccagtttgcaaaaggtggaaaatgatacatccccacaccgtgaaagagccactttgctggaggagcagctgcccctagggaaggcctcgttccacatacctcaagtccaagtgagggacgaaggacagtaccaatgcataatcatctatggggtcgcctgggactacaagtacctgactctgaaagtcaaagcttcctacaggaaaataaacactcacatcctaaaggttccagaaacagatgaggtagagctcacctgccaggctacaggttatcctctggcagaagtatcctggccaaacgtcagcgttcctgccaacaccagccactccaggacccctgaaggcctctaccaggtcaccagtgttctgcgcctaaagccaccccctggcagaaacttcagctgtgtgttctggaatactcacgtgagggaacttactttggccagcattgaccttcaaagtcagatggaacccaggacccatccaactggcggagggggaagtggcgggggtgggtccggcggcggcggctcgggtgctgctcctctgaagattcaagcttatttcaatgagactgcagacctgccatgccaatttgcaaactctcaaaaccaaagcctgagtgagctagtagtattttggcaggaccaggaaaacttggttctgaatgaggtatacttaggcaaagagaaatttgacagtgttcattccaagtatatgggccgcacaagttttgattcggacagttggaccctgagacttcacaatcttcagatcaaggacaagggcttgtatcaatgtatcatccatcacaaaaagcccacaggaatgattcgcatccaccagatgaattctgaactgtcagtgcttgctaacttcagtcaacctgaaatagtaccaatttctaatataacagaaaatgtgtacataaatttgacctgctcatctatacacggttacccagaacctaagaagatgagtgttttgctaagaaccaagaattcaactatcgagtatgatggtattatgcagaaatctcaagataatgtcacagaactgtacgacgtttccatcagcttgtctgtttcattccctgatgttacgagcaatatgaccatcttctgtattctggaaactgacaagacgcggcttttatcttcacctttctctatagagcttgaggaccctcagcctcccccagaccacattcct

SEQ ID NO: 12 - protein, 254 aa, Artificial Sequence
  vector
MGWSCIILFLVATATGVHSEIVLTQSPATLSLSPGERATLSCRASQSVSSYLAWYQQKPGQAPRLLIYDASNRATGIPARFSGSGSGTDFTLTISSLEPEDFAVYYCQQRSNWPTFGQGTKVEIKSGGGGSQVQLVQSGAEVKKPGSSVKVSCKTSGDTFSTYAISWVRQAPGQGLEWMGGIIPIFGKAHYAQKFQGRVTITADESTSTAYMELSSLRSEDTAVYFCARKFHFVSGSPFGMDVWGQGTTVTVSS

SEQ ID NO: 13 - protein, 253 aa, Artificial Sequence
  vector
MGWSCIILFLVATATGVHSAIQLTQSPSSLSASVGDRVTITCRASQGISSALAWYQQKPGKAPKLLIYDASSLESGVPSRFSGSGSGTDFTLTISSLQPEDFATYYCQQFNSYPFTFGPGTKVDIKSGGGGSEVQLVESGGGLVQPGRSLRLSCAASGITFDDYGMHWVRQAPGKGLEWVSGISWNRGRIEYADSVKGRFTISRDNAKNSLYLQMNSLRAEDTALYYCAKGRFRYFDWFLDYWGQGTLVTVSS

SEQ ID NO: 14 - protein, 254 aa, Artificial Sequence
  vector
MGWSCIILFLVATATGVHSEIVLTQSPATLSLSPGERATLSCRASQSVSSYLAWYQQKPGQAPRLLIYDASNRATGIPARFSGSGSGTDFTLTISSLEPEDFAVYYCQQRSNWPTFGQGTKVEIKSGGGGSQVQLVQSGAEVKKPGSSVKVSCKTSGDTFSSYAISWVRQAPGQGLEWMGGIIPIFGRAHYAQKFQGRVTITADESTSTAYMELSSLRSEDTAVYFCARKFHFVSGSPFGMDVWGQGTTVTVSS

SEQ ID NO: 15 - protein, 250 aa, Artificial Sequence
  vector
MGWSCIILFLVATATGVHSDIQMTQSPSSLSASVGDRVTITCRASQGISSWLAWYQQKPEKAPKSLIYAASSLQSGVPSRFSGSGSGTDFTLTISSLQPEDFATYYCQQYNSYPYTFGQGTKLEIKSGGGGSQVQLVQSGAEVKKPGASVKVSCKASGYTFTSYDVHWVRQAPGQRLEWMGWLHADTGITKFSQKFQGRVTITRDTSASTAYMELSSLRSEDTAVYYCARERIQLWFDYWGQGTLVTVSS

SEQ ID NO: 16 - protein, 249 aa, Artificial Sequence
  vector
MGWSCIILFLVATATGVHSEIVLTQSPATLSLSPGERATLSCRASQSVSSYLVWYQQKPGQAPRLLIYDASNRATGIPARFSGSGSGTDFTLTISSLEPEDFAVYYCQQRSNWPRTFGQGTKVEIKSGGGGSQVQLVQSGAEVKKPGASVKVSCKASGYTFTDYGFSWVRQAPGQGLEWMGWITAYNGNTNYAQKLQGRVTMTTDTSTSTVYMELRSLRSDDTAVYYCARDYFYGMDVWGQGTTVTVSS

SEQ ID NO: 17 - protein, 250 aa, Artificial Sequence
  vector
GGGGSQVQLVQSGAEVKKPGASVKVSCKASGYTFTSYYIHWVRQAPGQGLEWIGCIYPGNVNTNYNEKFKDRATLTVDTSISTAYMELSRLRSDDTAVYFCTRSHYGLDWNFDVWGQGTTVTVSSVEGGSGGSGGSGGSGGVDDIQMTQSPSSLSASVGDRVTITCHASQNIYVWLNWYQQKPGKAPKLLIYKASNLHTGVPSRFSGSGSGTDFTLTISSLQPEDFATYYCQQGQTYPYTFGGGTKVEIK